European Patent Application EP 4 424 700 A1, published September 4, 2024. Title: 수지상 세포를 표적하는 신규한 펩타이드, 및 이를 포함하는 암 치료용 조성물. Applicant: 전남대학교산학협력단. The sequence listing filed with the application follows.

SEQUENCE LISTING (25 sequences)

SEQ ID NO: 1 - protein, 14 aa, synthetic construct
  REGION 1..14: note = peptide 1
ARPGVSMRIEAHGG

SEQ ID NO: 2 - protein, 13 aa, synthetic construct
  REGION 1..13: note = peptide 2
ARQYNGIFHPVRS

SEQ ID NO: 3 - protein, 14 aa, synthetic construct
  REGION 1..14: note = peptide 3
SPACLDLGLVPWRI

SEQ ID NO: 4 - protein, 14 aa, synthetic construct
  REGION 1..14: note = peptide 4
VDLYPCYTFHSRVV

SEQ ID NO: 5 - protein, 14 aa, synthetic construct
  REGION 1..14: note = peptide 5
HFAWRTILWGTTHH

SEQ ID NO: 6 - protein, 14 aa, synthetic construct
  REGION 1..14: note = peptide 6, and DCpep6
RFFCLGPLGFTKVD

SEQ ID NO: 7 - protein, 14 aa, synthetic construct
  REGION 1..14: note = DCpep1
ARPGVSMKIEAHGG

SEQ ID NO: 8 - protein, 13 aa, synthetic construct
  REGION 1..13: note = DCpep2
ARQYNGIFHPVKS

SEQ ID NO: 9 - protein, 14 aa, synthetic construct
  REGION 1..14: note = DCpep3
SPACLDLGLVPWKI

SEQ ID NO: 10 - protein, 14 aa, synthetic construct
  REGION 1..14: note = DCpep4
VDLYPCYTFHSKVV

SEQ ID NO: 11 - protein, 14 aa, synthetic construct
  REGION 1..14: note = DCpep5
HFAWKTILWGTTHH

SEQ ID NO: 12 - DNA, 31 bp, synthetic construct
  misc_feature 1..31: note = E7-F (NdeI)
  source 1..31: mol_type = other DNA
gggaattccatatgcatggtgacacgcccac

SEQ ID NO: 13 - DNA, 27 bp, synthetic construct
  misc_feature 1..27: note = E7-R (XhoI)
  source 1..27: mol_type = other DNA
ccgctcgagtggtttctgggagcatat

SEQ ID NO: 14 - DNA, 32 bp, synthetic construct
  misc_feature 1..32: note = E7deltaNLS-F (NdeI)
  source 1..32: mol_type = other DNA
gggaattccatatgatcgatgggccggccggt

SEQ ID NO: 15 - DNA, 27 bp, synthetic construct
  misc_feature 1..27: note = E7deltaNLS-R (XhoI)
  source 1..27: mol_type = other DNA
ccgctcgagtggtttctgggagcatat

SEQ ID NO: 16 - DNA, 29 bp, synthetic construct
  misc_feature 1..29: note = E7deltaNLS-F (EcoRI)
  source 1..29: mol_type = other DNA
ccggaattcaattggatcgatgtacgcta

SEQ ID NO: 17 - DNA, 27 bp, synthetic construct
  misc_feature 1..27: note = E7deltaNLS-R (HindIII)
  source 1..27: mol_type = other DNA
cccaagctttggtttctgggagcatat

SEQ ID NO: 18 - DNA, 29 bp, synthetic construct
  misc_feature 1..29: note = FlaB-F (HindIII)
  source 1..29: mol_type = other DNA
cccaagcttatggcagtgaatgtaaatac

SEQ ID NO: 19 - DNA, 29 bp, synthetic construct
  misc_feature 1..29: note = FlaB-R (XhoI)
  source 1..29: mol_type = other DNA
ccgctcgaggcctagtagacttagcgctg

SEQ ID NO: 20 - DNA, 35 bp, synthetic construct
  misc_feature 1..35: note = DCpep6-F (NdeI)
  source 1..35: mol_type = other DNA
gggaattccatatgcgcttcttctgtttgggtcca

SEQ ID NO: 21 - protein, 105 aa, synthetic construct
  REGION 1..105: note = E7FL
MHGDTPTLHEYMLDLQPETTDLYCYEQLNDSSEEEDEIDGPAGQAEPDRAHYNIVTFCCKCDSTLRLCVQSTVDIRTLEDLLMGTLGIVCPICSQKPLEHHHHHH

SEQ ID NO: 22 - protein, 70 aa, synthetic construct
  REGION 1..70: note = E7deltaNLS (E)
MIDGPAGQAEPDRAHYNIVTFCCKCDSTLRLCVQSTHVDIRTLEDLLMGTLGIVCPICSQKPLEHHHHHH

SEQ ID NO: 23 - protein, 377 aa, synthetic construct
  REGION 1..377: note = FlaB (F)
MAVNVNTNVAAMTAQRYLNNANSAQQTSMERLSSGFKINSAKDDAAGLQISNRLNVQSRGLDVAVRNANDGISIAQTAEGAMNETTNILQRMRDLSLQSANGSNSKSERVAIQEEVTALNDELNRIAETTSFGGNKLLNGTYGTKAMQIGADNGEAVMLSLKDMRSDNVMMGGVSYQAEEGKDKNWNVAAGDNDLTIALTDSFGNEQEIEINAKAGDDIEELATYINGQTDLVKASVGEGGKLQIFAGNNKVQGEIAFSGSLAGELGLGEGKNVTVDTIDVTTVQGAQESVAIVDAALKYVDSHRAELGAFQNRFNHAISNLDNINENVNASKSRIKDTDFAKETTQLTKTQILSQASSSILAQAKQAPNSALSLLG

SEQ ID NO: 24 - protein, 638 aa, synthetic construct
  REGION 1..638: note = 4xE7deltaNLS::FlaB (EF)
MIDGPAGQAEPDRAHYNIVTFCCKCDSTLRLCVQSTHVDIRTLEDLLMGTLGIVCPICSQKPEFIDGPAGQAEPDRAHYNIVTFCCKCDSTLRLCVQSTHVDIRTLEDLLMGTLGIVCPICSQKPVDIDGPAGQAEPDRAHYNIVTFCCKCDSTLRLCVQSTHVDIRTLEDLLMGTLGIVCPICSQKPVDIDGPAGQAEPDRAHYNIVTFCCKCDSTLRLCVQSTHVDIRTLEDLLMGTLGIVCPICSQKPKLMAVNVNTNVAAMTAQRYLNNANSAQQTSMERLSSGFKINSAKDDAAGLQISNRLNVQSRGLDVAVRNANDGISIAQTAEGAMNETTNILQRMRDLSLQSANGSNSKSERVAIQEEVTALNDELNRIAETTSFGGNKLLNGTYGTKAMQIGADNGEAVMLSLKDMRSDNVMMGGVSYQAEEGKDKNWNVAAGDNDLTIALTDSFGNEQEIEINAKAGDDIEELATYINGQTDLVKASVGEGGKLQIFAGNNKVQGEIAFSGSLAGELGLGEGKNVTVDTIDVTTVQGAQESVAIVDAALKYVDSHRAELGAFQNRFNHAISNLDNINENVNASKSRIKDTDFAKETTQLTKTQILSQASSSILAQAKQAPNSALSLLGLEHHHHHH

SEQ ID NO: 25 - protein, 652 aa, synthetic construct
  REGION 1..652: note = DCpep6::4xE7deltaNLS::FlaB (DEF)
MRFFCLGPLGFTKVDIDGPAGQAEPDRAHYNIVTFCCKCDSTLRLCVQSTHVDIRTLEDLLMGTLGIVCPICSQKPEFIDGPAGQAEPDRAHYNIVTFCCKCDSTLRLCVQSTHVDIRTLEDLLMGTLGIVCPICSQKPVDIDGPAGQAEPDRAHYNIVTFCCKCDSTLRLCVQSTHVDIRTLEDLLMGTLGIVCPICSQKPVDIDGPAGQAEPDRAHYNIVTFCCKCDSTLRLCVQSTHVDIRTLEDLLMGTLGIVCPICSQKPKLMAVNVNTNVAAMTAQRYLNNANSAQQTSMERLSSGFKINSAKDDAAGLQISNRLNVQSRGLDVAVRNANDGISIAQTAEGAMNETTNILQRMRDLSLQSANGSNSKSERVAIQEEVTALNDELNRIAETTSFGGNKLLNGTYGTKAMQIGADNGEAVMLSLKDMRSDNVMMGGVSYQAEEGKDKNWNVAAGDNDLTIALTDSFGNEQEIEINAKAGDDIEELATYINGQTDLVKASVGEGGKLQIFAGNNKVQGEIAFSGSLAGELGLGEGKNVTVDTIDVTTVQGAQESVAIVDAALKYVDSHRAELGAFQNRFNHAISNLDNINENVNASKSRIKDTDFAKETTQLTKTQILSQASSSILAQAKQAPNSALSLLGLEHHHHHH